European Patent Specification EP 4 259 647 B1, published July 1, 2026. Title: COMPOSITIONS AND METHODS FOR THE TREATMENT OF METABOLIC AND LIVER DISORDERS. Applicant: Viking Therapeutics, Inc. Application WO. The sequence listing filed with the application follows.

SEQUENCE LISTING (47 sequences)

SEQ ID NO: 1 - protein, 16 aa, synthetic construct
  VARIANT 2: note = wherein X is 2-aminoisobutyric acid
  VARIANT 13: note = wherein X can be 2-aminoisobutyric acid, any naturally occurring amino acid, or any unnaturally occurring amino acid
  VARIANT 16: note = wherein X is -(A)n1-(B)n2-(C)n3-(D)n4-; wherein A, B, C, and D are independently any naturally occurring amino acid, or any unnaturally occurring amino acid; wherein each of n1, n2, n3, and n4 are independently 0 or 1
YXEGTFTSDYSIXLDX

SEQ ID NO: 2 - protein, 20 aa, unidentified
  VARIANT 1: note = wherein X is -(A)n1-(B)n2-(C)n3-(D)n4-; wherein A, B, C, and D are independently any naturally occurring amino acid, or any unnaturally occurring amino acid; wherein each of n1, n2, n3, and n4 are independently 0 or 1
  VARIANT 5: note = wherein X can be any naturally occurring amino acid, any unnaturally occurring amino acid, or 2-aminoisobutyric acid
  VARIANT 9: note = wherein X can be 2-aminoisobutyric acid, any naturally occurring amino acid, or any unnaturally occurring amino acid
XAFVXWLIXGGPSSGAPPPS

SEQ ID NO: 3 - protein, 19 aa, synthetic construct
  NON_STD 2: note = wherein X is 2-aminoisobutyric acid
  VARIANT 13: note = wherein X is 2-aminoisobutyric acid
YXEGTFTSDYSIXLDKIAQ

SEQ ID NO: 4 - protein, 19 aa, synthetic construct
AFVQWLIAGGPSSGAPPPS

SEQ ID NO: 5 - protein, 7 aa, synthetic construct
KVAKIAQ

SEQ ID NO: 6 - protein, 4 aa, synthetic construct
KTAQ

SEQ ID NO: 7 - protein, 4 aa, synthetic construct
KTSQ

SEQ ID NO: 8 - protein, 4 aa, synthetic construct
KVAQ

SEQ ID NO: 9 - protein, 4 aa, synthetic construct
RIAQ

SEQ ID NO: 10 - protein, 4 aa, synthetic construct
KIAK

SEQ ID NO: 11 - protein, 4 aa, synthetic construct
KISQ

SEQ ID NO: 12 - protein, 4 aa, synthetic construct
IAQQ

SEQ ID NO: 13 - protein, 4 aa, synthetic construct
IAQK

SEQ ID NO: 14 - protein, 4 aa, synthetic construct
VAQK

SEQ ID NO: 15 - protein, 15 aa, synthetic construct
  NON_STD 2: note = wherein X is 2-aminoisobutyric acid
  NON_STD 13: note = wherein X is 2-aminoisobutyric acid
YXEGTFTSDYSIXLD

SEQ ID NO: 16 - protein, 23 aa, synthetic construct
IAQQAFVQWLIAGGPSSGAPPPS

SEQ ID NO: 17 - protein, 19 aa, synthetic construct
  NON_STD 2: note = wherein X is 2-aminoisobutyric acid
  NON_STD 13: note = wherein X is 2-aminoisobutyric acid
YXEGTFTSDYSIXLDRIAQ

SEQ ID NO: 18 - protein, 19 aa, synthetic construct
AFVQWLIAGGPSSGAPPPS

SEQ ID NO: 19 - protein, 19 aa, synthetic construct
  NON_STD 2: note = wherein X is 2-aminoisobutyric acid
  NON_STD 13: note = wherein X is 2-aminoisobutyric acid
YXEGTFTSDYSIXLDKVAQ

SEQ ID NO: 20 - protein, 19 aa, synthetic construct
  VARIANT 2: note = wherein X is 2-aminoisobutyric acid
YXEGTFTSDYSIFLDKIAQ

SEQ ID NO: 21 - protein, 19 aa, synthetic construct
  NON_STD 2: note = wherein X is 2-aminoisobutyric acid
YXEGTFTSDYSIFLDKVAQ

SEQ ID NO: 22 - protein, 19 aa, synthetic construct
  NON_STD 2: note = wherein X is 2-aminoisobutyric acid
  NON_STD 13: note = wherein X is 2-aminoisobutyric acid
YXEGTFTSDYSIXLDKIAQ

SEQ ID NO: 23 - protein, 19 aa, synthetic construct
AFVQWLIRGGPSSGAPPPS

SEQ ID NO: 24 - protein, 19 aa, synthetic construct
  VARIANT 2: note = wherein X is 2-aminoisobutyric acid
YXEGTFTSDYSIFLDKIAQ

SEQ ID NO: 25 - protein, 19 aa, synthetic construct
AFVNWLIAGGPSSGAPPPS

SEQ ID NO: 26 - protein, 18 aa, synthetic construct
  NON_STD 2: note = wherein X is 2-aminoisobutyric acid
  NON_STD 13: note = wherein X is 2-aminoisobutyric acid
YXEGTFTSDYSIXLDKIA

SEQ ID NO: 27 - protein, 20 aa, synthetic construct
QAFVNWLIAGGPSSGAPPPS

SEQ ID NO: 28 - protein, 19 aa, synthetic construct
  NON_STD 2: note = wherein X is 2-aminoisobutyric acid
  NON_STD 13: note = wherein X is 2-aminoisobutyric acid
YXEGTFTSDYSIXLDKTAQ

SEQ ID NO: 29 - protein, 19 aa, synthetic construct
  NON_STD 2: note = wherein X is 2-aminoisobutyric acid
  NON_STD 13: note = wherein X is 2-aminoisobutyric acid
YXEGTFTSDYSIXLDKISQ

SEQ ID NO: 30 - protein, 19 aa, synthetic construct
  NON_STD 2: note = wherein X is 2-aminoisobutyric acid
  NON_STD 13: note = wherein X is 2-aminoisobutyric acid
YXEGTFTSDYSIXLDKIAQ

SEQ ID NO: 31 - protein, 19 aa, synthetic construct
AFVQWLIAGGPSSGAPPPS

SEQ ID NO: 32 - protein, 15 aa, synthetic construct
  NON_STD 2: note = wherein X is 2-aminoisobutyric acid
  NON_STD 13: note = wherein X is 2-aminoisobutyric acid
YXEGTFTSDYSIXLD

SEQ ID NO: 33 - protein, 23 aa, synthetic construct
IAQQAFVQWLIAGGPSSGAPPPS

SEQ ID NO: 34 - protein, 19 aa, synthetic construct
  NON_STD 2: note = wherein X is 2-aminoisobutyric acid
  NON_STD 13: note = wherein X is 2-aminoisobutyric acid
YXEGTFTSDYSIXLDRIAQ

SEQ ID NO: 35 - protein, 19 aa, synthetic construct
  NON_STD 2: note = wherein X is 2-aminoisobutyric acid
  NON_STD 13: note = wherein X is 2-aminoisobutyric acid
YXEGTFTSDYSIXLDKVAQ

SEQ ID NO: 36 - protein, 19 aa, synthetic construct
  NON_STD 2: note = wherein X is 2-aminoisobutyric acid
YXEGTFTSDYSIFLDKIAQ

SEQ ID NO: 37 - protein, 19 aa, synthetic construct
  NON_STD 2: note = wherein X is 2-aminoisobutyric acid
YXEGTFTSDYSIFLDKVAQ

SEQ ID NO: 38 - protein, 19 aa, synthetic construct
  VARIANT 2: note = wherein X is 2-aminoisobutyric acid
  NON_STD 13: note = wherein X is 2-aminoisobutyric acid
YXEGTFTSDYSIXLDKIAQ

SEQ ID NO: 39 - protein, 19 aa, synthetic construct
AFVQWLIRGGPSSGAPPPS

SEQ ID NO: 40 - protein, 19 aa, synthetic construct
  VARIANT 2: note = wherein X is 2-aminoisobutyric acid
YXEGTFTSDYSIFLDKIAQ

SEQ ID NO: 41 - protein, 19 aa, synthetic construct
AFVNWLIAGGPSSGAPPPS

SEQ ID NO: 42 - protein, 19 aa, synthetic construct
  VARIANT 2: note = wherein X is 2-aminoisobutyric acid
  NON_STD 13: note = wherein X is 2-aminoisobutyric acid
YXEGTFTSDYSIXLDKTAQ

SEQ ID NO: 43 - protein, 19 aa, synthetic construct
  VARIANT 2: note = wherein X is 2-aminoisobutyric acid
  NON_STD 13: note = wherein X is 2-aminoisobutyric acid
YXEGTFTSDYSIXLDKISQ

SEQ ID NO: 44 - protein, 18 aa, synthetic construct
  VARIANT 2: note = wherein X is 2-aminoisobutyric acid
  NON_STD 13: note = wherein X is 2-aminoisobutyric acid
YXEGTFTSDYSIXLDKIA

SEQ ID NO: 45 - protein, 20 aa, synthetic construct
QAFVNWLIAGGPSSGAPPPS

SEQ ID NO: 46 - protein, 19 aa, synthetic construct
  VARIANT 2: note = wherein X is 2-aminoisobutyric acid
  NON_STD 13: note = wherein X is 2-aminoisobutyric acid
YXEGTFTSDYSIXLDKVAQ

SEQ ID NO: 47 - protein, 19 aa, synthetic construct
AFVQWLIRGGPSSGAPPPS